European Patent Application EP 4 455 278 A1, published October 30, 2024. Title: Glycosyltransferase mutant and method of preparing steviol glycosides using the same. Applicant: SAMYANG CORPORATION. The sequence listing filed with the application follows.

SEQUENCE LISTING (30 sequences)

SEQ ID NO: 1 - protein, 461 aa, synthetic construct
  REGION 1..461: note = TaUGT wild-type Glycosyltransferase
MDDGSSSSSSPLRVVICPWLAFGHLLPCLDIAERLASRGHRVSFVSTPRNIARLPPVRPAVAPLVDYVALPLPRVDGLPEGAESTNDVPHDKFELLRKAFDGLAAPFSEFLHAACAEGTGKRPDWLIVDSFHHWAAAAAVENKVPCVMLLLGAANVIATWARGVSEHAAAAVGKERSAAEAPSFETERRKLMITQNASGMTVAERYFLTLMRSNLVAIRSCAEWEPESVAALTTLAGKPVVTLGLLPPSPEGGRGISKQDAAVRWLDAQRDKSVVYVALGSEVPLRVEQVHELALGLELSGASFLWALRKPPGMPDAAVLPPGFEERTRGRGLVVTGWVPQISVLAHGAVAAFLTHCGWNSTIEGLLFGQPLIMLPISSDQGPNARLMEGRKVGMQVPRNESDGSFTREDVAATVQAVAMEEDGSRVFTANAKTMQEIVADSACHERCIDGFIQQLRSYKE

SEQ ID NO: 2 - DNA, 1383 bp, synthetic construct
  misc_feature 1..1383: note = TaUGT wild-type Glycosyltransferase
  source 1..1383: mol_type = other DNA
atggacgacgggtcttctagctctagcagtccgctgcgtgttgttatttgcccgtggctggcttttggacacctgcttccatgcttagacattgcggaaagattagccagccgtggacacagagtatccttcgtaagtacgccgcgtaatatagcacgtttacccccggtcagaccggcagttgcgccgctggtcgattacgtagcgctacctctgcccagagtggacggacttccggaaggggctgaatctacaaacgacgtgccccatgataagttcgagcttttacgtaaggctttcgacggtttggcagcgcccttcagcgaatttctacacgcagcgtgcgcggagggcacaggcaaaagaccagattggcttattgtggattccttccaccattgggctgcggctgcggcagtggaaaataaagtcccgtgcgtcatgttacttttaggtgcagccaacgtgatcgccacttgggcacgtggcgtgtcagagcatgcggccgccgcggttggaaaagaacgtagtgccgcagaagctccatcattcgaaaccgaacgtcgtaaactgatgataactcagaatgcatcaggtatgaccgtagcagagcgttatttcctgacacttatgagatcaaacttggttgccattcgttcctgtgcagaatgggagcctgaatctgtggcggcactaaccactctggccgggaagcccgtagtgaccttaggtttgcttccaccgtctcctgagggaggaaggggtatttccaagcaagacgctgccgttaggtggctggacgctcagagggataagtccgttgtatacgtggcgttagggtctgaagttcccttgagagtggagcaggtacatgagcttgcgcttggactagagttgtcaggtgctagcttcctgtgggcgttacgtaagccacccggcatgcctgacgccgcagtcttgccgccgggttttgaagagagaaccaggggacgtggtctggttgtgactggctgggtaccacaaatcagcgtcttagcacatggcgccgttgccgcttttctgacacattgcggctggaatagtacaatcgaaggcttgctgttcggacaaccgttaatcatgctgccaatcagtagcgatcagggcccgaatgcccgtcttatggagggaagaaaagttggaatgcaggtgcctcgtaatgagtccgatggatcattcacaagagaggatgtcgctgccacagtacaagcagtagcgatggaggaggatgggagccgtgtttttacggctaatgcaaagaccatgcaagaaatagttgctgactccgcgtgtcacgaaaggtgcatcgatggatttatccaacagctaaggtcctataaagaa

SEQ ID NO: 3 - protein, 461 aa, synthetic construct
  REGION 1..461: note = TaUGT mutant Glycosyltransferase
MDDGSSSSSSPLRVVICPWLAFGHLLPCLDIAERLASRGHRVSFVSTPRNIARLPPVRPAVAPLVDYVALPLPRVDGLPEGAESTNDVPHDKFELLRKAFDGLAAPFSEFLHAACAEGTGKRPDWLIVDSFHHWAAAAAVENKVPCVMLLLGAANVIATWARGVSEHAAAAVGKERSAAEAPSFETERRKLMITQNASGMSLAERYFLTLMRSNLVAIRSCAEWEPESVAALTTLAGKPVVTLGLLPPSPEGGRGISKQDAAVRWLDAQRDKSVVYVALGSEVPLRVEQVHELALGLELSGASFLWALRKPPGMPDAAVLPPGFEERTRGRGLVVTGWVPQISVLAHGAVAAFLTHCGWNSTIEGLLFGQPLIMLPISSDQGPNARLMEGRKVGMQVPRNESDGSFTREDVAATVQAVAMEEDGSRVFTANAKTMQEIVADSACHERCIDGFIQQLRSYKE

SEQ ID NO: 4 - protein, 808 aa, synthetic construct
  REGION 1..808: note = SUS(Arabidopsis thaliana SUS1)
MANAERMITRVHSQRERLNETLVSERNEVLALLSRVEAKGKGILQQNQIIAEFEALPEQTRKKLEGGPFFDLLKSTQEAIVLPPWVALAVRPRPGVWEYLRVNLHALVVEELQPAEFLHFKEELVDGVKNGNFTLELDFEPFNASIPRPTLHKYIGNGVDFLNRHLSAKLFHDKESLLPLLKFLRLHSHQGKNLMLSEKIQNLNTLQHTLRKAEEYLAELKSETLYEEFEAKFEEIGLERGWGDNAERVLDMIRLLLDLLEAPDPCTLETFLGRVPMVFNVVILSPHGYFAQDNVLGYPDTGGQVVYILDQVRALEIEMLQRIKQQGLNIKPRILILTRLLPDAVGTTCGERLERVYDSEYCDILRVPFRTEKGIVRKWISRFEVWPYLETYTEDAAVELSKELNGKPDLIIGNYSDGNLVASLLAHKLGVTQCTIAHALEKTKYPDSDIYWKKLDDKYHFSCQFTADIFAMNHTDFIITSTFQEIAGSKETVGQYESHTAFTLPGLYRVVHGIDVFDPKFNIVSPGADMSIYFPYTEEKRRLTKFHSEIEELLYSDVENKEHLCVLKDKKKPILFTMARLDRVKNLSGLVEWYGKNTRLRELANLVVVGGDRRKESKDNEEKAEMKKMYDLIEEYKLNGQFRWISSQMDRVRNGELYRYICDTKGAFVQPALYEAFGLTVVEAMTCGLPTFATCKGGPAEIIVHGKSGFHIDPYHGDQAADTLADFFTKCKEDPSHWDEISKGGLQRIEEKYTWQIYSQRLLTLTGVYGFWKHVSNLDRLEARRYLEMFYALKYRPLAQAVPLAQDD

SEQ ID NO: 5 - DNA, 2424 bp, synthetic construct
  misc_feature 1..2424: note = SUS(Arabidopsis thaliana SUS1)
  source 1..2424: mol_type = other DNA
atggctaacgccgaacgtatgatcacgagggtacactcccaacgtgaacgtttaaatgaaactttggtcagcgagcgtaacgaggttctagcactactttccagggtcgaagctaaggggaaggggatacttcagcaaaatcagataatcgcggagttcgaggctttaccggagcagaccagaaaaaagttagagggtggcccgttctttgatctacttaaatctacacaggaggctattgtgctgccaccttgggtcgccctggcagtcaggcctaggccaggcgtatgggagtaccttcgtgttaatttgcacgcattagtagtggaggaattacagcctgccgaatttctacactttaaagaggagttagtggacggtgtcaagaatggaaacttcacccttgagcttgatttcgaaccattcaatgccagcataccccgtcctacattacacaaatatattgggaacggggtcgactttctgaataggcatctatcagctaagttgttccatgacaaggaatcccttcttcctctattgaaatttttgagacttcacagtcatcaggggaagaacttgatgttaagcgagaaaatacaaaacttgaatacgttacaacatacgcttagaaaggcagaggagtatctggcggaactaaagagtgagactttgtacgaagagttcgaagccaagtttgaggaaataggtcttgaacgtgggtggggcgacaatgctgaacgtgtcctggatatgatacgtcttttactggacttattagaggcaccggacccatgtaccctagaaacattcttagggagggtacccatggttttcaacgttgtcattcttagtccgcatggatattttgcccaagataacgtgttaggataccccgacaccgggggacaagttgtttatattttagatcaagtaagagcattagagattgagatgttacaaagaattaaacagcagggtctgaacataaaaccaaggatcttaattttgactcgtcttcttcctgatgcagtggggacgacgtgcggagagaggctggaacgtgtctacgattcagaatattgtgatatcctgagagtgccctttagaacagaaaaaggaatcgtgcgtaagtggatcagtagatttgaagtctggccatatctggagacatacaccgaagatgcagcggtcgaacttagcaaagagctaaacgggaaacccgacctgataatcgggaactacagcgacgggaatttagttgccagtttacttgcccataagctgggagtgacacagtgcacgatagcccacgcccttgaaaagacgaagtatcccgattctgacatatattggaaaaaacttgatgacaaataccatttttcatgccaattcactgctgatatctttgcaatgaatcacacggatttcatcattacttccacatttcaagagatcgcaggcagcaaagagacagttggacaatatgagagtcatactgcattcacactacctggtctttatagagtcgtgcacggtatagacgtgtttgatcctaagttcaacatagtctcaccgggtgcggatatgtccatctactttccctacactgaggaaaagaggcgtttaaccaagtttcattcagagatagaagagttattatatagtgatgtggaaaataaagagcatctatgcgtgttaaaagacaagaagaaacctatcctattcacaatggccagacttgacagagtgaagaatctatccggcttggttgaatggtacggcaagaacacgcgtcttcgtgagctagcgaaccttgtcgtagtaggaggtgacagaagaaaggaatccaaagacaacgaagagaaagcggagatgaaaaagatgtacgatctaatcgaagaatacaaattaaatggtcagttccgttggatctcctctcagatggatagagtccgtaatggagaactatacagatatatatgcgacaccaaaggcgcgtttgtgcagccggcattgtacgaggcctttggtctgactgtcgtcgaggccatgacctgcggccttcctacattcgcgacctgcaaaggtggtccagctgagattattgtccatgggaaatctggattccacatagacccatatcatggtgaccaggccgctgatacacttgcagatttttttactaagtgtaaggaggacccttcacattgggatgaaatatccaaagggggactgcagcgtatcgaggagaaatatacctggcaaatatatagccaaaggctgttgaccctaacgggcgtttacgggttctggaagcacgtttccaatctagataggctagaggcgaggcgttacctggaaatgttttacgcgttgaaatacaggcctctagcacaagcagtaccactggcgcaggacgat

SEQ ID NO: 6 - protein, 1275 aa, synthetic construct
  REGION 1..1275: note = Amino acid sequence of fused protein
MDDGSSSSSSPLRVVICPWLAFGHLLPCLDIAERLASRGHRVSFVSTPRNIARLPPVRPAVAPLVDYVALPLPRVDGLPEGAESTNDVPHDKFELLRKAFDGLAAPFSEFLHAACAEGTGKRPDWLIVDSFHHWAAAAAVENKVPCVMLLLGAANVIATWARGVSEHAAAAVGKERSAAEAPSFETERRKLMITQNASGMSLAERYFLTLMRSNLVAIRSCAEWEPESVAALTTLAGKPVVTLGLLPPSPEGGRGISKQDAAVRWLDAQRDKSVVYVALGSEVPLRVEQVHELALGLELSGASFLWALRKPPGMPDAAVLPPGFEERTRGRGLVVTGWVPQISVLAHGAVAAFLTHCGWNSTIEGLLFGQPLIMLPISSDQGPNARLMEGRKVGMQVPRNESDGSFTREDVAATVQAVAMEEDGSRVFTANAKTMQEIVADSACHERCIDGFIQQLRSYKEGGGGSGMANAERMITRVHSQRERLNETLVSERNEVLALLSRVEAKGKGILQQNQIIAEFEALPEQTRKKLEGGPFFDLLKSTQEAIVLPPWVALAVRPRPGVWEYLRVNLHALVVEELQPAEFLHFKEELVDGVKNGNFTLELDFEPFNASIPRPTLHKYIGNGVDFLNRHLSAKLFHDKESLLPLLKFLRLHSHQGKNLMLSEKIQNLNTLQHTLRKAEEYLAELKSETLYEEFEAKFEEIGLERGWGDNAERVLDMIRLLLDLLEAPDPCTLETFLGRVPMVFNVVILSPHGYFAQDNVLGYPDTGGQVVYILDQVRALEIEMLQRIKQQGLNIKPRILILTRLLPDAVGTTCGERLERVYDSEYCDILRVPFRTEKGIVRKWISRFEVWPYLETYTEDAAVELSKELNGKPDLIIGNYSDGNLVASLLAHKLGVTQCTIAHALEKTKYPDSDIYWKKLDDKYHFSCQFTADIFAMNHTDFIITSTFQEIAGSKETVGQYESHTAFTLPGLYRVVHGIDVFDPKFNIVSPGADMSIYFPYTEEKRRLTKFHSEIEELLYSDVENKEHLCVLKDKKKPILFTMARLDRVKNLSGLVEWYGKNTRLRELANLVVVGGDRRKESKDNEEKAEMKKMYDLIEEYKLNGQFRWISSQMDRVRNGELYRYICDTKGAFVQPALYEAFGLTVVEAMTCGLPTFATCKGGPAEIIVHGKSGFHIDPYHGDQAADTLADFFTKCKEDPSHWDEISKGGLQRIEEKYTWQIYSQRLLTLTGVYGFWKHVSNLDRLEARRYLEMFYALKYRPLAQAVPLAQDD

SEQ ID NO: 7 - protein, 4 aa, synthetic construct
  REGION 1..4: note = Linker for fused protein
GGGS

SEQ ID NO: 8 - protein, 5 aa, synthetic construct
  REGION 1..5: note = Linker for fused protein
GGGGS

SEQ ID NO: 9 - protein, 9 aa, synthetic construct
  REGION 1..9: note = Linker for fused protein
GGGSGGGGS

SEQ ID NO: 10 - protein, 15 aa, synthetic construct
  REGION 1..15: note = Linker for fused protein
GGGGSGGGGSGGGGS

SEQ ID NO: 11 - protein, 12 aa, synthetic construct
  REGION 1..12: note = Linker for fused protein
GGGGPSPGGGGS

SEQ ID NO: 12 - protein, 462 aa, synthetic construct
  REGION 1..462: note = EUGT11 enzyme
MDSGYSSSYAAAAGMHVVICPWLAFGHLLPCLDLAQRLASRGHRVSFVSTPRNISRLPPVRPALAPLVAFVALPLPRVEGLPDGAESTNDVPHDRPDMVELHRRAFDGLAAPFSEFLGTACADWVIVDVFHHWAAAAALEHKVPCAMMLLGSAHMIASIADRRLERAETESPAAAGQGRPAAAPTFEVARMKLIRTKGSSGMSLAERFSLTLSRSSLVVGRSCVEFEPETVPLLSTLRGKPITFLGLMPPLHEGRREDGEDATVRWLDAQPAKSVVYVALGSEVPLGVEKVHELALGLELAGTRFLWALRKPTGVSDADLLPAGFEERTRGRGVVATRWVPQMSILAHAAVGAFLTHCGWNSTIEGLMFGHPLIMLPIFGDQGPNARLIEAKNAGLQVARNDGDGSFDREGVAAAIRAVAVEEESSKVFQAKAKKLQEIVADMACHERYIDGFIQQLRSYKD

SEQ ID NO: 13 - DNA, 1386 bp, synthetic construct
  misc_feature 1..1386: note = EUGT11 enzyme
  source 1..1386: mol_type = other DNA
atggactccggctacagttcatcatatgctgcagccgctgggatgcacgttgtgatttgtccgtggctagcattcggtcatctgttgccgtgtttggacctggctcagaggctagcttccagaggacatcgtgtttccttcgtttctacgcctaggaatatcagtagactaccaccggtaagacctgctttagctccacttgtggcgttcgtggccctaccgttaccccgtgtagaaggattgcctgacggagcagagtctacgaatgacgtacctcacgacagacccgatatggttgaacttcacagaagagcgttcgacggtcttgctgcaccgttttccgaattccttgggacggcctgtgcggactgggtcatagtggacgtattccatcactgggctgccgcagctgccctagaacataaggttccgtgtgccatgatgttgttaggttctgctcatatgatcgcgtctattgcagaccgtaggttggagagggcagaaacggaaagtccagccgccgccggacaggggaggcccgctgcggcgccaacctttgaggtggctcgtatgaaactaattaggactaaaggttcaagcggtatgtcactggcggaaaggtttagtcttactttgtccaggtcttcattggtcgtcggtcgttcctgcgttgagtttgaacccgaaaccgttccccttctttccacgttacgtggaaaaccgattacttttcttggtcttatgccgccactgcacgagggtagaagggaagatggtgaagacgctacagttaggtggctagacgcgcaaccggctaagagcgtcgtctatgtcgcacttggctcagaggtgcccttgggggtcgagaaggtccatgagttggcgctggggttggagttggcgggtacaaggtttctttgggcccttcgtaaaccgacgggcgtatcagatgcagacctacttccggctggtttcgaggagcgtactaggggaaggggcgttgtggccacgagatgggtgccacaaatgagcatcctagctcatgccgcagtcggcgcattcttaacgcattgtggctggaattcaaccattgaagggctaatgttcggtcatccactgataatgcttcctatctttggagaccaaggtcccaatgcgcgtttgatcgaagccaagaatgctggccttcaagtcgcccgtaatgatggcgatggttcattcgacagagagggagtggcggcagcgatcagagcggttgcagtggaagaggagtccagtaaggtgtttcaggctaaggccaagaaattacaggagatagtggctgatatggcttgccacgagagatatatcgacggctttatacaacagctacgttcttataaggac

SEQ ID NO: 14 - protein, 463 aa, synthetic construct
  REGION 1..463: note = HvUGT enzyme
MDGDGNSSSSSSPLHVVICPWLALGHLLPCLDIAERLASRGHRVSFVSTPRNIARLPPLRPAVAPLVEFVALPLPHVDGLPEGAESTNDVPYDKFELHRKAFDGLAAPFSEFLRAACAEGAGSRPDWLIVDTFHHWAAAAAVENKVPCVMLLLGAATVIAGFARGVSEHAAAAVGKERPAAEAPSFETERRKLMTTQNASGMTVAERYFLTLMRSDLVAIRSCAEWEPESVAALTTLAGKPVVPLGLLPPSPEGGRGVSKEDAAVRWLDAQPAKSVVYVALGSEVPLRAEQVHELALGLELSGARFLWALRKPTDAPDAAVLPPGFEERTRGRGLVVTGWVPQIGVLAHGAVAAFLTHCGWNSTIEGLLFGHPLIMLPISSDQGPNARLMEGRKVGMQVPRDESDGSFRREDVAATVRAVAVEEDGRRVFTANAKKMQEIVADGACHERCIDGFIQQLRSYKA

SEQ ID NO: 15 - DNA, 1389 bp, synthetic construct
  misc_feature 1..1389: note = HvUGT enzyme
  source 1..1389: mol_type = other DNA
atggacggcgacggaaacagttcatcaagttctagtcctctgcatgttgttatatgtccctggctagctcttgggcatcttcttccttgtttggacattgcggaaagactggcctcaagaggacacagggtcagcttcgtatccacgccaagaaatattgcccgtctacccccgcttaggccagcggtggctcccttagtagagttcgttgctctacctctgcctcacgtggacgggttacctgaaggggctgaaagtacaaacgatgtaccctatgacaagtttgaacttcaccgtaaggcgttcgacgggctggccgctccttttagcgagttcttgagagctgcttgtgccgagggggctggttcccgtcctgattggctaatcgtggatacattccatcactgggcagcggcagccgccgttgaaaataaagtgccatgcgtgatgttactgcttggtgcagccaccgttattgccgggttcgcaagaggggtcagtgagcacgccgccgctgcagtcggtaaagagagaccggccgctgaagccccgagttttgagacggagagacgtaaacttatgaccactcagaatgcaagtggtatgacggttgcagaaaggtatttcctaaccttaatgcgtagtgacttggtcgcaatacgtagctgcgccgagtgggagcccgagtctgtcgcggcgttgacaaccttagcaggcaagcccgtcgttcctttaggcttgctgccaccgtctccagagggggggagaggcgtttccaaggaggacgccgcggttcgttggttggatgcgcaacccgcgaagagcgtcgtgtatgtcgcgttaggcagtgaggttccattgagagctgaacaagtccacgagttggcgcttggtttagaattatctggcgctaggtttttatgggcgctaaggaaacccaccgacgcgccagatgccgcggtattgccgccagggtttgaggaaaggactcgtggcagagggcttgtcgtgaccggttgggtgcctcaaatcggcgttcttgctcatggtgccgtagcagcattcttgactcattgtggctggaattcaaccatcgaggggctgctgtttggtcacccgttgatcatgctgccaataagctccgaccaaggacccaatgctcgtttgatggaaggcagaaaagtggggatgcaggtgcccagagacgaaagcgatgggagttttaggagagaagatgtggcagctactgttcgtgctgtagcggtggaggaagatggcagaagggtttttacagctaatgcgaagaagatgcaagaaatagtagccgacggggcttgtcacgagagatgcatcgatggatttatccaacaactgcgttcctacaaagct

SEQ ID NO: 16 - DNA, 28 bp, synthetic construct
  misc_feature 1..28: note = Reverse promoter of GAL10 promoter
  source 1..28: mol_type = other DNA
catcaattcttactttttttttggatgg

SEQ ID NO: 17 - DNA, 31 bp, synthetic construct
  misc_feature 1..31: note = Forward terminator of CYC1 terminator
  source 1..31: mol_type = other DNA
tgattgtcgatatcatgtaattagttatgtc

SEQ ID NO: 18 - DNA, 44 bp, synthetic construct
  misc_feature 1..44: note = Forward promoter of TaUGT connecting GAL10 promoter
  source 1..44: mol_type = other DNA
catccaaaaaaaaagtaagaattgatggacgacgggtcttctag

SEQ ID NO: 19 - DNA, 48 bp, synthetic construct
  misc_feature 1..48: note = Reverse promoter of TaUGT connecting CYC1 terminator
  source 1..48: mol_type = other DNA
ctaattacatgatatcgacaatcattctttataggaccttagctgttg

SEQ ID NO: 20 - DNA, 44 bp, synthetic construct
  misc_feature 1..44: note = Forward promoter of EUGT11 connecting GAL10 promoter
  source 1..44: mol_type = other DNA
catccaaaaaaaaagtaagaattgatggactccggctacagttc

SEQ ID NO: 21 - DNA, 45 bp, synthetic construct
  misc_feature 1..45: note = Reverse promoter of EUGT11 connecting CYC1 terminator
  source 1..45: mol_type = other DNA
ctaattacatgatatcgacaattagtccttataagaacgtagctg

SEQ ID NO: 22 - DNA, 42 bp, synthetic construct
  misc_feature 1..42: note = Forward promoter of HvUGT connecting GAL10 promoter
  source 1..42: mol_type = other DNA
catccaaaaaaaaagtaagaattgatggacggcgacggaaac

SEQ ID NO: 23 - DNA, 45 bp, synthetic construct
  misc_feature 1..45: note = Reverse promoter of HvUGT connecting CYC1 terminator
  source 1..45: mol_type = other DNA
ctaattacatgatatcgacaatcaagctttgtaggaacgcagttg

SEQ ID NO: 24 - DNA, 32 bp, synthetic construct
  misc_feature 1..32: note = Forward promoter for mutant T201S or V202L of TaUGT
  source 1..32: mol_type = other DNA
caggtatgtcwbtagcagagcgttatttcctg

SEQ ID NO: 25 - DNA, 34 bp, synthetic construct
  misc_feature 1..34: note = Reverse promoter for mutant T201S or V202L of TaUGT
  source 1..34: mol_type = other DNA
cgctctgctavwgacatacctgatgcattctgag

SEQ ID NO: 26 - DNA, 44 bp, synthetic construct; identical to SEQ ID NO: 18
  misc_feature 1..44: note = Forward promoter for mutant TaUGT
  source 1..44: mol_type = other DNA

SEQ ID NO: 27 - DNA, 43 bp, synthetic construct
  misc_feature 1..43: note = Reverse promoter for mutant TaUGT-LInker
  source 1..43: mol_type = other DNA
tccactaccaccgccaccttctttataggaccttagctgttgg

SEQ ID NO: 28 - DNA, 39 bp, synthetic construct
  misc_feature 1..39: note = Forward promoter for linker-SUS
  source 1..39: mol_type = other DNA
ggtggcggtggtagtggaatggctaacgccgaacgtatg

SEQ ID NO: 29 - DNA, 42 bp, synthetic construct
  misc_feature 1..42: note = Reverse promoter for SUS
  source 1..42: mol_type = other DNA
ctaattacatgatatcgacaattactcggcagccagagggac

SEQ ID NO: 30 - DNA, 1383 bp, synthetic construct
  misc_feature 1..1383: note = TaUGT mutant Glycosyltransferase
  source 1..1383: mol_type = other DNA
atggacgacgggtcttctagctctagcagtccgctgcgtgttgttatttgcccgtggctggcttttggacacctgcttccatgcttagacattgcagaaagattagccagccgtggacacagagtatccttcgtaagtacgccgcgtaatatagcacgtttacccccggtcagaccggcagttgcgccgctggtcgattacgtagcgctacctctgcccagagtggacggacttccggaaggggctgaatctacaaacgacgtgccccatgataagttcgagcttttacgtaaggctttcgacggtttggcagcgcccttcagcgaatttctacacgcagcgtgcgcggagggcacaggcaaaagaccagattggcttattgtggattccttccaccattgggctgcggctgcggcagtggaaaataaagtcccgtgcgtcatgttacttttaggtgcagccaacgtgatcgccacttgggcacgtggcgtgtcagagcatgcggccgccgcggttggaaaagaacgtagtgccgcagaagctccatcattcgaaaccgaacgtcgtaaactgatgataactcagaatgcatcaggtatgtcattagcagagcgttatttcctgacacttatgagatcaaacttggttgccattcgttcctgtgcagaatgggagcctgaatctgtggcggcactaaccactctggccgggaagcccgtagtgaccttaggtttgcttccaccgtctcctgagggaggaaggggtatttccaagcaagacgctgccgttaggtggctggacgctcagagggataagtccgttgtatacgtggcgttagggtctgaagttcccttgagagtggagcaggtacatgagcttgcgcttggactagagttgtcaggtgctagcttcctgtgggcgttacgtaagccacccggcatgcctgacgccgcagtcttgccgccgggttttgaagagagaaccaggggacgtggtctggttgtgactggctgggtaccacaaatcagcgtcttagcacatggcgccgttgccgcttttctgacacattgcggctggaatagtacaatcgaaggcttgctgttcggacaaccgttaatcatgctgccaatcagtagcgatcagggcccgaatgcccgtcttatggagggaagaaaagttggaatgcaggtgcctcgtaatgagtccgatggatcattcacaagagaggatgtcgctgccacagtacaagcagtagcgatggaggaggatgggagccgtgtttttacggctaatgcaaagaccatgcaagaaatagttgctgactccgcgtgtcacgaaaggtgcatcgatggatttatccaacagctaaggtcctataaagaa